European Patent Specification EP 3 744 834 B1, published September 10, 2025. Title: SYNTHETIC OPLOPHORUS LUCIFERASES WITH ENHANCED LIGHT OUTPUT. Applicant: Promega Corporation. The sequence listing filed with the application follows.

SEQUENCE LISTING (32 sequences)

SEQ ID NO: 1 - protein, 169 aa, Oplophorus gracilirostris
FTLADFVGDWQQTAGYNQDQVLEQGGLSSLFQALGVSVTPIQKVVLSGENGLKADIHVIIPYEGLSGFQMGLIEMIFKVVYPVDDHHFKIILHYGTLVIDGVTPNMIDYFGRPYPGIAVFDGKQITVTGTLWNGNKIYDERLINPDGSLLFRVTINGVTGWRLCENILA

SEQ ID NO: 2 - DNA, 513 bp, Artificial Sequence
  Synthetic
atggtgtttaccttggcagatttcgttggagactggcaacagacagctggatacaaccaagatcaagtgttagaacaaggaggattgtctagtctgttccaagccctgggagtgtcagtcaccccaatccagaaagttgtgctgtctggggagaatgggttaaaagctgatattcatgtcatcatcccttacgagggactcagtggttttcaaatgggtctgattgaaatgatcttcaaagttgtttacccagtggatgatcatcatttcaagattattctccattatggtacactcgttattgacggtgtgacaccaaacatgattgactactttggacgcccttaccctggaattgctgtgtttgacggcaagcagatcacagttactggaactctgtggaacggcaacaagatctatgatgagcgcctgatcaacccagatggttcactcctcttccgcgttactatcaatggagtcaccggatggcgcctttgcgagaacattcttgcc

SEQ ID NO: 3 - protein, 131 aa, Bos taurus
SNKFLGTWKLVSSENFDEYMKALGVGLATRKLGNLAKPRVIISKKGDIITIRTESPFKNTEISFKLGQEFEETTADNRKTKSTVTLARGSLNQVQKWNGNETTIKRKLVDGKMVVECKMKDVVCTRIYEKV

SEQ ID NO: 4 - protein, 134 aa, Rattus rattus
PVDFNGYWKMLSNENFEEYLRALDVNVALRKIANLLKPDKEIVQDGDHMIIRTLSTFRNYIMDFQVGKEFEEDLTGIDDRKCMTTVSWDGDKLQCVQKGEKEGRGWTQWIEGDELHLEMRAEGVTCKQVFKKVH

SEQ ID NO: 5 - protein, 135 aa, Schistosoma mansoni
GSMSSFLGKWKLSESHNFDAVMSKLGVSWATRQIGNTVTPTVTFTMDGDKMTMLTESTFKNLSCTFKFGEEFDEKTSDGRNVKSVVEKNSESKLTQTQVDPKNTTVIVREVDGDTMKTTVTVGDVTAIRNYKRLS

SEQ ID NO: 6 - protein, 135 aa, Schistosoma mansoni; identical to SEQ ID NO: 5

SEQ ID NO: 7 - protein, 165 aa, Artificial Sequence
  Synthetic
LADFVGDWQQTAGYNQDQVLEQGGLSSLFQALGVSVTPIQKVVLSGENGLKADIHVIIPYEGLSGFQMGLIEMIFKVVYPVDDHHFKIILHYGTLVIDGVTPNMIDYFGRPYPGIAVFDGKQITVTGTLWNGNKIYDERLINPDGSLLFRVTINGVTGWRLCENI

SEQ ID NO: 8 - protein, 131 aa, Bos taurus; identical to SEQ ID NO: 3

SEQ ID NO: 9 - protein, 134 aa, Rattus rattus; identical to SEQ ID NO: 4

SEQ ID NO: 10 - protein, 196 aa, Oplophorus gracilirostris
MAYSTLFIIALTAVVTQASSTQKSNLTFTLADFVGDWQQTAGYNQDQVLEQGGLSSLFQALGVSVTPIQKVVLSGENGLKADIHVIIPYEGLSGFQMGLIEMIFKVVYPVDDHHFKIILHYGTLVIDGVTPNMIDYFGRPYPGIAVFDGKQITVTGTLWNGNKIYDERLINPDGSLLFRVTINGVTGWRLCENILA

SEQ ID NO: 11 - protein, 131 aa, Bos taurus; identical to SEQ ID NO: 3

SEQ ID NO: 12 - DNA, 588 bp, Oplophorus gracilirostris
atggcgtactccactctgttcataattgcattgaccgccgttgtcactcaagcttcctcaactcaaaaatctaacctaacttttacgttggcagatttcgttggagactggcaacagacagctggatacaaccaagatcaagtgttagaacaaggaggattgtctagtctgttccaagccctgggagtgtcagtcacgcccatacagaaagttgtactgtctggggagaatgggttaaaagctgatattcatgtcataataccttacgagggactcagtggttttcaaatgggtctaattgaaatgatcttcaaagttgtttaccccgtggatgatcatcatttcaagattattctccattatggtacactcgttattgacggtgtaacacccaacatgattgactactttggaagaccttaccctggaattgctgtatttgacggcaagcagatcacagttactggaactctgtggaacggcaacaagatctatgatgagaggctaatcaaccctgatggttcactcctcttcagagttactatcaatggagtcacgggatggaggctttgcgagaacattcttgcc

SEQ ID NO: 13 - protein, 171 aa, Artificial Sequence
  Synthetic
MVFTLADFVGDWQQTAGYNQDQVLEQGGLSSLFQALGVSVTPIQKVVLSGENGLKADIHVIIPYEGLSGFQMGLIEMIFKVVYPVDDHHFKIILHYGTLVIDGVTPNMIDYFGRPYPGIAVFDGKQITVTGTLWNGNKIYDERLINPDGSLLFRVTINGVTGWRLCENILA

SEQ ID NO: 14 - DNA, 513 bp, Artificial Sequence
  Synthetic
atggtgtttaccttggcagatttcgttggagactggcaacagacagctggatacaaccaagatcaagtgttagaacaaggaggattgtctagtctgttccaagccctgggagtgtcagtcaccccaatccagaaagttgtgctgtctggggagaatgggttaaaagctgatattcatgtcatcatcccttacgagggactcagtggttttcaaatgggtctgattgaaatgatcttcaaagttgtttacccagtggatgatcatcatttcaagattattctccattatggtacactcgttattgacggtgtgacaccaaacatgattgactactttggacgcccttaccctggaattgctgtgtttgacggcaagcagatcacagttactggaactctgtggaacggcaacaagatctatgatgagcgcctgatcaacccagatggttcactcctcttccgcgttactatcaatggagtcaccggatggcgcctttgcgagcgtattcttgcc

SEQ ID NO: 15 - protein, 171 aa, Artificial Sequence
  Synthetic
MVFTLADFVGDWQQTAGYNQDQVLEQGGLSSLFQALGVSVTPIQKVVLSGENGLKADIHVIIPYEGLSGFQMGLIEMIFKVVYPVDDHHFKIILHYGTLVIDGVTPNMIDYFGRPYPGIAVFDGKQITVTGTLWNGNKIYDERLINPDGSLLFRVTINGVTGWRLCERILA

SEQ ID NO: 16 - DNA, 513 bp, Artificial Sequence
  Synthetic
atggtgtttacattggaggatttcgttggagactggcggcagacagctggatacaaccaagatcaagtgttagaacaaggaggattgtctagtctgttccaaaagctgggagtgtcagtcaccccaatccagaaaattgtgctgtctggggagaatgggttaaaatttgatattcatgtcatcatcccttacgagggactcagtggttttcaaatgggtctgattgaaatgatcttcaaagttgtttacccagtggatgatcatcatttcaagattattctccattatggtacactcgttattgacggtgtgacaccaaacatgattgactactttggacgcccttacgagggaattgctgtgtttgacggcaagaagatcacagttactggaactctgtggaacggcaacaagatcattgatgagcgcctgatcaacccagatggttcactcctcttccgcgttactatcaatggagtcaccggatggcgcctttgcgagcgtattcttgcc

SEQ ID NO: 17 - protein, 133 aa, Locusta migratoria
VKEFAGIKYKLDSQTNFEEYMKAIGVGAIERKAGLALSPVIELEVLDGDKFKLTSKTAIKNTEFTFKLGEEFDEDTLDGRKVKSIITQDGPNKLVHEQKGDHPTIIIREFSKEQCVITIKLGDLVATRIYKAQ

SEQ ID NO: 18 - protein, 125 aa, Bufo arenarum
AFNGTWNVYAQENYENFLRTVGLPEDIIKVAKDVNPVIEIEQNGNEFVVTSKTPKQTHSNSFTVGKESEITSMDGKKIKVTVQLEGGKLICKSDKFSHIQEVNGDEMVEKITIGSSTLTRKSKRV

SEQ ID NO: 19 - protein, 134 aa, Echinococcus granulosus
  misc_feature (1)..(1): Xaa can be any naturally occurring amino acid
  misc_feature (64)..(64): Xaa can be any naturally occurring amino acid
XMEAFLGTWKMEKSEGFDKIMERLGVDFVTRKMGNLVKPNLIVTDLGGGKYKMRSESTFKTTEXSFKLGEKFKEVTPDSREVASLITVENGVMKHEQDDKTKVTYIERVVEGNELKATVKVDEVVCVRTYSKVA

SEQ ID NO: 20 - protein, 190 aa, Mycobacterium tuberculosis
AAVERAKATAARNIPAFDDLPVPADTANLREGADLNNALLALLPLVGVWRGEGEGRGPDGDYRFGQQIVVSHDGGDYLNWESRSWRLTATGDYQEPGLREAGFWRFVAIELLLAHSAGYVELFYGRPRTQSSWELVTDALARSRSGVLVGGAKRLYGIVEGGDLAYVEERVDADGGLVPHLSARLSRFVG

SEQ ID NO: 21 - protein, 351 aa, Lingulodinium polyedrum
  misc_feature (31)..(31): Xaa can be any naturally occurring amino acid
  misc_feature (45)..(45): Xaa can be any naturally occurring amino acid
  misc_feature (90)..(90): Xaa can be any naturally occurring amino acid
  misc_feature (123)..(123): Xaa can be any naturally occurring amino acid
  misc_feature (203)..(203): Xaa can be any naturally occurring amino acid
  misc_feature (265)..(265): Xaa can be any naturally occurring amino acid
  misc_feature (286)..(286): Xaa can be any naturally occurring amino acid
EKGFEAGDNKLGGALNAKHVEKYGDNFKNGXHKPEFHEDGLHKPXEVGGKKFESGFHYLLECHELGGKNASGGYGGPLCEDPYGSEVQAXTEKLLKEADSDRTLCFNNFQDPCPQLTKEQVAXCKGFDYGDKTLKLPCGPLPWPAGLPEPGYVPKTNPLHGRWITVSGGQAAFIKEAIKSGMLGAAEANKIVADTDHHQTGGXYLRINQFGDVCTVDASVAKFARAKRTWKSGHYFYEPLVSGGNLLGVWVLPEEYRKIGFFWEXESGRCFRIERRAFPVGPYTFXRQATEVGGKISFVFYVKVSNDPESDPIPLQSRDYTALAGRDNAPTNLGKPYPTLAKDLDYPKKRD

SEQ ID NO: 22 - protein, 131 aa, Homo sapiens
VDAFLGTWKLVDSKNFDDYMKSLGVGFATRQVASMTKPTTIIEKNGDILTLKTHSTFKNTEISFKLGVEFDETTADDRKVKSIVTLDGGKLVHLQKWDGQETTLVRELIDGKLILTLTHGTAVCTRTYEKE

SEQ ID NO: 23 - protein, 171 aa, Artificial Sequence
  Synthetic
MVFTLEDFVGDWRQTAGYNQDQVLEQGGLSSLFQKLGVSVTPIQKIVLSGENGLKFDIHVIIPYEGLSGFQMGLIEMIFKVVYPVDDHHFKIILHYGTLVIDGVTPNMIDYFGRPYEGIAVFDGKKITVTGTLWNGNKIIDERLINPDGSLLFRVTINGVTGWRLCERILA

SEQ ID NO: 24 - DNA, 513 bp, Artificial Sequence
  Synthetic
atggtgtttacattggcagatttcgttggagactggcggcagacagctggatacaaccaagatcaagtgttagaacaaggaggattgtctagtctgttccaaaagctgggagtgtcagtcaccccaatccagaaaattgtgctgtctggggagaatgggttaaaatttgatattcatgtcatcatcccttacgagggactcagtggttttcaaatgggtctgattgaaatgatcttcaaagttgtttacccagtggatgatcatcatttcaagattattctccattatggtacactcgttattgacggtgtgacaccaaacatgattgactactttggacgcccttacgagggaattgctgtgtttgacggcaagaagatcacagttactggaactctgtggaacggcaacaagatcattgatgagcgcctgatcaacccagatggttcactcctcttccgcgttactatcaatggagtcaccggatggcgcctttgcgagcgtattcttgcc

SEQ ID NO: 25 - protein, 171 aa, Artificial Sequence
  Synthetic
MVFTLADFVGDWRQTAGYNQDQVLEQGGLSSLFQKLGVSVTPIQKIVLSGENGLKFDIHVIIPYEGLSGFQMGLIEMIFKVVYPVDDHHFKIILHYGTLVIDGVTPNMIDYFGRPYEGIAVFDGKKITVTGTLWNGNKIIDERLINPDGSLLFRVTINGVTGWRLCERILA

SEQ ID NO: 26 - DNA, 513 bp, Artificial Sequence
  Synthetic
atggtgtttacattggcagatttcgttggagactggcggcagacagctggatacaaccaagatcaagtgttagaacaaggaggattgtctagtctgttccaaaagctgggagtgtcagtcaccccaatccagaaaattgagctgtctggggagaatgggttaaaatttgatattcatgtcatcatcccttacgagggactcagtggttttcaaatgggtctgattgaaatgatcttcaaagttgtttacccagtggatgatcatcatttcaagattattctccattatggtacactcgttattgacggtgtgacacttaacatgattgactactttggacgcccttacgagggaattgctgtgtttgacggcaagaagatcacagttactggaactctgtggaacggcaagaagatcattgaggagcgcctgatcaacccagatggttcactcctcttccgcgttactatcaatggagtcaccggatggcgcctttgcgagcgtgttcttgcc

SEQ ID NO: 27 - protein, 171 aa, Artificial Sequence
  Synthetic
MVFTLADFVGDWRQTAGYNQDQVLEQGGLSSLFQKLGVSVTPIQKIELSGENGLKFDIHVIIPYEGLSGFQMGLIEMIFKVVYPVDDHHFKIILHYGTLVIDGVTLNMIDYFGRPYEGIAVFDGKKITVTGTLWNGKKIIEERLINPDGSLLFRVTINGVTGWRLCERVLA

SEQ ID NO: 28 - DNA, 513 bp, Artificial Sequence
  Synthetic
atggtgtttacattggaggatttcgttggagactggcggcagacagctggatacaaccaagatcaagtgttagaacaaggaggattgtctagtctgttccaaaagctgggagtgtcagtcaccccaatccagaaaattgagctgtctggggagaatgggttaaaatttgatattcatgtcatcatcccttacgagggactcagtggttttcaaatgggtctgattgaaatgatcttcaaagttgtttacccagtggatgatcatcatttcaagattattctccattatggtacactcgttattgacggtgtgacacttaacatgattgactactttggacgcccttacgagggaattgctgtgtttgacggcaagaagatcacagttactggaactctgtggaacggcaagaagatcattgaggagcgcctgatcaacccagatggttcactcctcttccgcgttactatcaatggagtcaccggatggcgcctttgcgagcgtgttcttgcc

SEQ ID NO: 29 - protein, 171 aa, Artificial Sequence
  Synthetic
MVFTLEDFVGDWRQTAGYNQDQVLEQGGLSSLFQKLGVSVTPIQKIELSGENGLKFDIHVIIPYEGLSGFQMGLIEMIFKVVYPVDDHHFKIILHYGTLVIDGVTLNMIDYFGRPYEGIAVFDGKKITVTGTLWNGKKIIEERLINPDGSLLFRVTINGVTGWRLCERVLA

SEQ ID NO: 30 - DNA, 513 bp, Artificial Sequence
  Synthetic
atggtgtttacattggaggatttcgttggagactggcggcagacagctggatacaaccaagatcaagtgttagaacaaggaggattgcctagtctgttccaaaagatgggagtgtcagtcaccccaatccagaaaattgtgctgtctggggagaatgtgttaaaatttgatattcatgtcatcatcccttacgagggactcagtggttttcaaatgggtctgattgaaatgatcttcaaagttgtttacccagtggatgatcatcatttcaagattattctccattatggtacactcgttgttgacggtgtgacaccaaacatgattgactactttggacgcccttacgagggaattgctgtgtttgacggcaagaagatcacagttactggaactctgtggaacggcaacaagatcattgatgagcgcctgctcaacccagatggttcactcctcttccgcgttactatcaatggagtcaccggatggcgcctttgcgagcgtattcttgcc

SEQ ID NO: 31 - protein, 171 aa, Artificial Sequence
  Synthetic
MVFTLEDFVGDWRQTAGYNQDQVLEQGGLPSLFQKMGVSVTPIQKIVLSGENVLKFDIHVIIPYEGLSGFQMGLIEMIFKVVYPVDDHHFKIILHYGTLVVDGVTPNMIDYFGRPYEGIAVFDGKKITVTGTLWNGNKIIDERLLNPDGSLLFRVTINGVTGWRLCERILA

SEQ ID NO: 32 - DNA, 513 bp, Artificial Sequence
  Synthetic
atggtgtttacattggcagatttcgttggagactggcaacagacagctggatacaaccaagatcaagtgttagaacaaggaggattgtctagtctgttccaagccctgggagtgtcagtcaccccaatccagaaagttgtgctgtctggggagaatgggttaaaagctgatattcatgtcatcatcccttacgagggactcagtggttttcaaatgggtctgattgaaatgatcttcaaagttgtttacccagtggatgatcatcatttcaagattattctccattatggtacactcgttattgacggtgtgacaccaaacatgattgactactttggacgcccttaccctggaattgctgtgtttgacggcaagcagatcacagttactggaactctgtggaacggcaacaagatctatgatgagcgcctgatcaacccagatggttcactcctcttccgcgttactatcaatggagtcaccggatggcgcctttgcgagaacattcttgcc